European Patent Specification EP 3 640 344 B1, published March 13, 2024. Title: DIRECT ELECTRON TRANSFER-TYPE OXIDOREDUCTASE-MODIFIED MOLECULAR RECOGNITION ELEMENT. Applicant: Arkray, Inc. Ultizyme International Ltd. The sequence listing filed with the application follows.

SEQUENCE LISTING (9 sequences)

SEQ ID NO: 1 - DNA, 3706 bp, Burkholderia cepacia
  CDS (258)..(761)
  CDS (764)..(2380)
  CDS (2386)..(3660)
aagctttctgtttgattgcacgcgattctaaccgagcgtctgtgaggcggaacgcgacatgcttcgtgtcgcacacgtgtcgcgccgacgacacaaaaatgcagcgaaatggctgatcgttacgaatggctgacacattgaatggactataaaaccattgtccgttccggaatgtgcgcgtacatttcaggtccgcgccgatttttgagaaatatcaagcgtggttttcccgaatccggtgttcgagagaaggaaacatgcacaacgacaacactccccactcgcgtcgccacggcgacgcagccgcatcaggcatcacgcggcgtcaatggttgcaaggcgcgctggcgctgaccgcagcgggcctcacgggttcgctgacattgcgggcgcttgcagacaaccccggcactgcgccgctcgatacgttcatgacgctttccgaatcgctgaccggcaagaaagggctcagccgcgtgatcggcgagcgcctgctgcaggcgctgcagaagggctcgttcaagacggccgacagcctgccgcagctcgccggcgcgctcgcgtccggttcgctgacgcctgaacaggaatcgctcgcactgacgatcctcgaggcctggtatctcggcatcgtcgacaacgtcgtgattacgtacgaggaagcattaatgttcggcgtcgtgtccgatacgctcgtgatccgttcgtattgccccaacaaacccggcttctgggccgacaaaccgatcgagaggcaagcctgatggccgataccgatacgcaaaaggccgacgtcgtcgtcgttggatcgggtgtcgcgggcgcgatcgtcgcgcatcagctcgcgatggcgggcaaggcggtgatcctgctcgaagcgggcccgcgcatgccgcgctgggaaatcgtcgagcgcttccgcaatcagcccgacaagatggacttcatggcgccgtacccgtcgagcccctgggcgccgcatcccgagtacggcccgccgaacgactacctgatcctgaagggcgagcacaagttcaactcgcagtacatccgcgcggtgggcggcacgacgtggcactgggccgcgtcggcgtggcgcttcattccgaacgacttcaagatgaagagcgtgtacggcgtcggccgcgactggccgatccagtacgacgatctcgagccgtactatcagcgcgcggaggaagagctcggcgtgtggggcccgggccccgaggaagatctgtactcgccgcgcaagcagccgtatccgatgccgccgctgccgttgtcgttcaacgagcagaccatcaagacggcgctgaacaactacgatccgaagttccatgtcgtgaccgagccggtcgcgcgcaacagccgcccgtacgacggccgcccgacttgttgcggcaacaacaactgcatgccgatctgcccgatcggcgcgatgtacaacggcatcgtgcacgtcgagaaggccgaacgcgccggcgcgaagctgatcgagaacgcggtcgtctacaagctcgagacgggcccggacaagcgcatcgtcgcggcgctctacaaggacaagacgggcgccgagcatcgcgtcgaaggcaagtatttcgtgctcgccgcgaacggcatcgagacgccgaagatcctgctgatgtccgcgaaccgcgatttcccgaacggtgtcgcgaacagctcggacatggtcggccgcaacctgatggaccatccgggcaccggcgtgtcgttctatgcgagcgagaagctgtggccgggccgcggcccgcaggagatgacgtcgctgatcggtttccgcgacggtccgttccgcgcgaccgaagcggcgaagaagatccacctgtcgaacctgtcgcgcatcgaccaggagacgcagaagatcttcaaggccggcaagctgatgaagcccgacgagctcgacgcgcagatccgcgaccgttccgcacgctacgtgcagttcgactgcttccacgaaatcctgccgcaacccgagaaccgcatcgtgccgagcaagacggcgaccgatgcgatcggcattccgcgccccgagatcacgtatgcgatcgacgactacgtgaagcgcggcgccgcgcatacgcgcgaggtctacgcgaccgccgcgaaggtgctcggcggcacggacgtcgtgttcaacgacgaattcgcgccgaacaatcacatcacgggctcgacgatcatgggcgccgatgcgcgcgactccgtcgtcgacaaggactgccgcacgttcgaccatccgaacctgttcatttcgagcagcgcgacgatgccgaccgtcggtaccgtaaacgtgacgctgacgatcgccgcgctcgcgctgcggatgtcggacacgctgaagaaggaagtctgaccgtgcggaaatctactctcactttcctcatcgccggctgcctcgcgttgccgggcttcgcgcgcgcggccgatgcggccgatccggcgctggtcaagcgcggcgaatacctcgcgaccgccggcgactgcatggcctgccacaccgtgaagggcggcaagccgtacgcgggcggccttggcatgccggtaccgatgctcggcaagatctacacgagcaacatcacgcccgatcccgatacgggcatcggcaaatggacgttcgaggacttcgagcgcgcggtgcggcacggcgtgtcgaagaacggcgacaacctgtatccggcgatgccgtacgtgtcgtacgcgaagatcacggacgacgacgtacgcgcgctgtacgcctacttcatgcacggcgtcgagccggtcaagcaggcgccgccgaagaacgagattcccgcgctgctcagcatgcgctggccgctgaagatctggaactggctgttcctgaaggacggcccgtaccagccgaagccgtcgcagagcgccgaatggaatcgcggcgcgtatctggtgcagggtctcgcgcactgcagcacgtgccacacgccgcgcggcatcgcgatgcaggagaagtcgctcgacgaaaccggcggcagcttcctcgcggggtcggtgctcgccggctgggacggctacaacatcacgtcggacccgaatgcggggatcggcagctggacgcagcagcagctcgtgcagtatttgcgcaccggcagcgtgccgggcgtcgcgcaggcggccgggccgatggccgaggcggtcgagcacagcttctcgaagatgaccgaagcggacatcggtgcgatcgccacgtacgtccgcacggtgccggccgttgccgacagcaacgcgaagcagccgcggtcgtcgtggggcaagccggccgaggacgggctgaagctgcgcggtgtcgcgctcgcgtcgtcgggcatcgatccggcgcggctgtatctcggcaactgcgcgacgtgccaccagatgcagggcaagggcacgccggacggctattacccgtcgctgttccacaactccaccgtcggcgcgtcgaatccgtcgaacctcgtgcaggtgatcctgaacggcgtgcagcgcaagatcggcagcgaggatatcgggatgcccgctttccgctacgatctgaacgacgcgcagatcgccgcgctgacgaactacgtgaccgcgcagttcggcaatccggcggcgaaggtgacggagcaggacgtcgcgaagctgcgctgacatagtcgggcgcgccgacacggcgcaaccgataggacaggag

SEQ ID NO: 2 - protein, 168 aa, Burkholderia cepacia
MHNDNTPHSRRHGDAAASGITRRQWLQGALALTAAGLTGSLTLRALADNPGTAPLDTFMTLSESLTGKKGLSRVIGERLLQALQKGSFKTADSLPQLAGALASGSLTPEQESLALTILEAWYLGIVDNVVITYEEALMFGVVSDTLVIRSYCPNKPGFWADKPIERQA

SEQ ID NO: 3 - protein, 539 aa, Burkholderia cepacia
MADTDTQKADVVVVGSGVAGAIVAHQLAMAGKAVILLEAGPRMPRWEIVERFRNQPDKMDFMAPYPSSPWAPHPEYGPPNDYLILKGEHKFNSQYIRAVGGTTWHWAASAWRFIPNDFKMKSVYGVGRDWPIQYDDLEPYYQRAEEELGVWGPGPEEDLYSPRKQPYPMPPLPLSFNEQTIKTALNNYDPKFHVVTEPVARNSRPYDGRPTCCGNNNCMPICPIGAMYNGIVHVEKAERAGAKLIENAVVYKLETGPDKRIVAALYKDKTGAEHRVEGKYFVLAANGIETPKILLMSANRDFPNGVANSSDMVGRNLMDHPGTGVSFYASEKLWPGRGPQEMTSLIGFRDGPFRATEAAKKIHLSNLSRIDQETQKIFKAGKLMKPDELDAQIRDRSARYVQFDCFHEILPQPENRIVPSKTATDAIGIPRPEITYAIDDYVKRGAAHTREVYATAAKVLGGTDVVFNDEFAPNNHITGSTIMGADARDSVVDKDCRTFDHPNLFISSSATMPTVGTVNVTLTIAALALRMSDTLKKEV

SEQ ID NO: 4 - protein, 425 aa, Burkholderia cepacia
MRKSTLTFLIAGCLALPGFARAADAADPALVKRGEYLATAGDCMACHTVKGGKPYAGGLGMPVPMLGKIYTSNITPDPDTGIGKWTFEDFERAVRHGVSKNGDNLYPAMPYVSYAKITDDDVRALYAYFMHGVEPVKQAPPKNEIPALLSMRWPLKIWNWLFLKDGPYQPKPSQSAEWNRGAYLVQGLAHCSTCHTPRGIAMQEKSLDETGGSFLAGSVLAGWDGYNITSDPNAGIGSWTQQQLVQYLRTGSVPGVAQAAGPMAEAVEHSFSKMTEADIGAIATYVRTVPAVADSNAKQPRSSWGKPAEDGLKLRGVALASSGIDPARLYLGNCATCHQMQGKGTPDGYYPSLFHNSTVGASNPSNLVQVILNGVQRKIGSEDIGMPAFRYDLNDAQIAALTNYVTAQFGNPAAKVTEQDVAKLR

SEQ ID NO: 5 - protein, 5 aa, Artificial Sequence
  linker
GGGGS

SEQ ID NO: 6 - protein, 7 aa, Artificial Sequence
  partial sequence
QDVAKLR

SEQ ID NO: 7 - protein, 4 aa, Artificial Sequence
  partial sequence
MASQ

SEQ ID NO: 8 - protein, 4 aa, Artificial Sequence
  partial sequence
DAAP

SEQ ID NO: 9 - protein, 8 aa, Artificial Sequence
  His tag
GSHHHHHH